European Patent Specification EP 3 953 475 B1, published January 21, 2026. Title: NUCLEIC ACID MAZZOCCHIO AND METHODS OF MAKING AND USE THEREOF. Applicant: The University of Hong Kong TANNER Julian Alexander Shiu, Simon Chi-Chin. The sequence listing filed with the application follows.

SEQUENCE LISTING (13 sequences)

SEQ ID NO: 1 - DNA, 155 bp, Artificial Sequence
  Synthetic sequence - strand 1
gataggccgagatctgaggatgctggctcacgccattggctcgcgaccccgtccgctagacgttatgcacaaggcgttgtcattagatgcttaggtgctcaggccgtaatgaggccgcttggctgcgttcctccgccgcttgggaacagccccgc

SEQ ID NO: 2 - DNA, 39 bp, Artificial Sequence
  Synthetic sequence - strand 2
tccagctctgcggacggggtcgcgagccattcgagggct

SEQ ID NO: 3 - DNA, 40 bp, Artificial Sequence
  Synthetic sequence - strand 3
tcgcctgtaatacgccttgtgcataacgtcttgccaaccc

SEQ ID NO: 4 - DNA, 46 bp, Artificial Sequence
  Synthetic sequence - strand 4
tgcccgtaccctggtgcacctaagcatctaatgactctgcggaaga

SEQ ID NO: 5 - DNA, 52 bp, Artificial Sequence
  Synthetic sequence - strand 5
taccccactttagcgatagcggcctcattacggcctgtgctacccgtacgga

SEQ ID NO: 6 - DNA, 69 bp, Artificial Sequence
  Synthetic sequence - strand 6
atcagtacgattggcgtgagccagcatcctctagcggcggaggaacgcagcctaggcggaactcttcgg

SEQ ID NO: 7 - DNA, 32 bp, Artificial Sequence
  Synthetic sequence - strand 7
tcgctaaagtggggtaccgaagagttccgcct

SEQ ID NO: 8 - DNA, 28 bp, Artificial Sequence
  Synthetic sequence - strand 8
gatctcggcctatcgcggggctgttccc

SEQ ID NO: 9 - DNA, 20 bp, Artificial Sequence
  Synthetic sequence - strand 9
tcgtactgatgagccctcga

SEQ ID NO: 10 - DNA, 16 bp, Artificial Sequence
  Synthetic sequence - strand 10
gagctggagggttggc

SEQ ID NO: 11 - DNA, 20 bp, Artificial Sequence
  Synthetic sequence - strand 11
ttacaggcgatcttccgcag

SEQ ID NO: 12 - DNA, 28 bp, Artificial Sequence
  Synthetic sequence - strand 12
ccagggtacgggcatccgtacgggtagc

SEQ ID NO: 13 - protein, 14 aa, Artificial Sequence
  Synthetic Peptide
  D-amino acid (1)..(14)
KLAKLAKKLAKLAK